European Patent Specification EP 3 598 984 B1, published April 10, 2024. Title: COMPOSITIONS AND METHODS TO TREATING HEMOGLOBINOPATHIES. Applicant: CHILDREN'S MEDICAL CENTER CORPORATION. Application PCT/US15/27527. The sequence listing filed with the application follows.

SEQUENCE LISTING (325 sequences)

SEQ ID NO: 1 - DNA, 64 bp, Artificial Sequence
  Description of Artificial Sequence: Synthetic oligonucleotide
acgctcgcacagaacactcatggattctccatgtggtagagaatccatgagtgttctgtgcgag

SEQ ID NO: 2 - DNA, 64 bp, Artificial Sequence
  Description of Artificial Sequence: Synthetic oligonucleotide
cgcactcgcacagaacactcatggattctctaccacatggagaatccatgagtgttctgtgcga

SEQ ID NO: 3 - DNA, 64 bp, Artificial Sequence
  Description of Artificial Sequence: Synthetic oligonucleotide
acgctccagaggatgacgattgtttactccatgtggtagagtaaacaatcgtcatcctctggag

SEQ ID NO: 4 - DNA, 64 bp, Artificial Sequence
  Description of Artificial Sequence: Synthetic oligonucleotide
cgcactccagaggatgacgattgtttactctaccacatggagtaaacaatcgtcatcctctgga

SEQ ID NO: 5 - DNA, 64 bp, Artificial Sequence
  Description of Artificial Sequence: Synthetic oligonucleotide
acgcttcggagactccagacaatcgcctccatgtggtagaggcgattgtctggagtctccgaag

SEQ ID NO: 6 - DNA, 64 bp, Artificial Sequence
  Description of Artificial Sequence: Synthetic oligonucleotide
cgcacttcggagactccagacaatcgcctctaccacatggaggcgattgtctggagtctccgaa

SEQ ID NO: 7 - DNA, 64 bp, Artificial Sequence
  Description of Artificial Sequence: Synthetic oligonucleotide
acgctttctcttgcaacacgcacagactccatgtggtagagtctgtgcgtgttgcaagagaaag

SEQ ID NO: 8 - DNA, 64 bp, Artificial Sequence
  Description of Artificial Sequence: Synthetic oligonucleotide
cgcactttctcttgcaacacgcacagactctaccacatggagtctgtgcgtgttgcaagagaaa

SEQ ID NO: 9 - DNA, 64 bp, Artificial Sequence
  Description of Artificial Sequence: Synthetic oligonucleotide
acgctacagtaccctggagaaacacactccatgtggtagagtgtgtttctccagggtactgtag

SEQ ID NO: 10 - DNA, 64 bp, Artificial Sequence
  Description of Artificial Sequence: Synthetic oligonucleotide
cgcactacagtaccctggagaaacacactctaccacatggagtgtgtttctccagggtactgta

SEQ ID NO: 11 - DNA, 64 bp, Artificial Sequence
  Description of Artificial Sequence: Synthetic oligonucleotide
acgctcaacaagatgaagagcaccaactccatgtggtagagttggtgctcttcatcttgttgag

SEQ ID NO: 12 - DNA, 64 bp, Artificial Sequence
  Description of Artificial Sequence: Synthetic oligonucleotide
cgcactcaacaagatgaagagcaccaactctaccacatggagttggtgctcttcatcttgttga

SEQ ID NO: 13 - DNA, 64 bp, Artificial Sequence
  Description of Artificial Sequence: Synthetic oligonucleotide
acgctgcgctcggagactccagacaactccatgtggtagagttgtctggagtctccgagcgcag

SEQ ID NO: 14 - DNA, 64 bp, Artificial Sequence
  Description of Artificial Sequence: Synthetic oligonucleotide
cgcactgcgctcggagactccagacaactctaccacatggagttgtctggagtctccgagcgca

SEQ ID NO: 15 - DNA, 64 bp, Artificial Sequence
  Description of Artificial Sequence: Synthetic oligonucleotide
acgctgcgcttctcttgcaacacgcactccatgtggtagagtgcgtgttgcaagagaagcgcag

SEQ ID NO: 16 - DNA, 64 bp, Artificial Sequence
  Description of Artificial Sequence: Synthetic oligonucleotide
cgcactgcgcttctcttgcaacacgcactctaccacatggagtgcgtgttgcaagagaagcgca

SEQ ID NO: 17 - DNA, 64 bp, Artificial Sequence
  Description of Artificial Sequence: Synthetic oligonucleotide
acgctgcgcacagtaccctggagaaactccatgtggtagagtttctccagggtactgtgcgcag

SEQ ID NO: 18 - DNA, 64 bp, Artificial Sequence
  Description of Artificial Sequence: Synthetic oligonucleotide
cgcactgcgcacagtaccctggagaaactctaccacatggagtttctccagggtactgtgcgca

SEQ ID NO: 19 - DNA, 20 bp, Artificial Sequence
  Description of Artificial Sequence: Synthetic oligonucleotide
taagcttgatatcgaattcc

SEQ ID NO: 20 - DNA, 20 bp, Artificial Sequence
  Description of Artificial Sequence: Synthetic oligonucleotide
gctctagaactagtggatcc

SEQ ID NO: 21 - DNA, 27 bp, Artificial Sequence
  Description of Artificial Sequence: Synthetic oligonucleotide
ttgccggcatggtgagcaagggcgagg

SEQ ID NO: 22 - DNA, 29 bp, Artificial Sequence
  Description of Artificial Sequence: Synthetic oligonucleotide
tagcggccgcttacttgtacagctcgtcc

SEQ ID NO: 23 - DNA, 22 bp, Artificial Sequence
  Description of Artificial Sequence: Synthetic oligonucleotide
cgctcgagcatgcatctagagg

SEQ ID NO: 24 - DNA, 36 bp, Artificial Sequence
  Description of Artificial Sequence: Synthetic oligonucleotide
ttgcggccgccggccgcgcttaatgcgccgctacag

SEQ ID NO: 25 - DNA, 57 bp, Artificial Sequence
  Description of Artificial Sequence: Synthetic oligonucleotide
cgcacagaacactcatggattctccatgtggtagagaatccatgagtgttctgtgcg

SEQ ID NO: 26 - DNA, 57 bp, Artificial Sequence
  Description of Artificial Sequence: Synthetic oligonucleotide
tcggagactccagacaatcgcctccatgtggtagaggcgattgtctggagtctccga

SEQ ID NO: 27 - DNA, 57 bp, Artificial Sequence
  Description of Artificial Sequence: Synthetic oligonucleotide
cctccaggcagctcaaagatcctccatgtggtagaggatctttgagctgcctggagg

SEQ ID NO: 28 - DNA, 57 bp, Artificial Sequence
  Description of Artificial Sequence: Synthetic oligonucleotide
ttctcttgcaacacgcacagactccatgtggtagagtctgtgcgtgttgcaagagaa

SEQ ID NO: 29 - DNA, 57 bp, Artificial Sequence
  Description of Artificial Sequence: Synthetic oligonucleotide
tcaggactaggtgcagaatgtctccatgtggtagagacattctgcacctagtcctga

SEQ ID NO: 30 - DNA, 57 bp, Artificial Sequence
  Description of Artificial Sequence: Synthetic oligonucleotide
gatcgagtgttgaataatgatctccatgtggtagagatcattattcaacactcgatc

SEQ ID NO: 31 - DNA, 57 bp, Artificial Sequence
  Description of Artificial Sequence: Synthetic oligonucleotide
cagtaccctggagaaacacatctccatgtggtagagatgtgtttctccagggtactg

SEQ ID NO: 32 - DNA, 57 bp, Artificial Sequence
  Description of Artificial Sequence: Synthetic oligonucleotide
cactgtccacaggagaagccactccatgtggtagagtggcttctcctgtggacagtg

SEQ ID NO: 33 - DNA, 57 bp, Artificial Sequence
  Description of Artificial Sequence: Synthetic oligonucleotide
acagtaccctggagaaacacactccatgtggtagagtgtgtttctccagggtactgt

SEQ ID NO: 34 - DNA, 57 bp, Artificial Sequence
  Description of Artificial Sequence: Synthetic oligonucleotide
gcgccgcacagaacactcatgctccatgtggtagagcatgagtgttctgtgcggcgc

SEQ ID NO: 35 - DNA, 57 bp, Artificial Sequence
  Description of Artificial Sequence: Synthetic oligonucleotide
gcgctcggagactccagacaactccatgtggtagagttgtctggagtctccgagcgc

SEQ ID NO: 36 - DNA, 57 bp, Artificial Sequence
  Description of Artificial Sequence: Synthetic oligonucleotide
gcgccctccaggcagctcaaactccatgtggtagagtttgagctgcctggagggcgc

SEQ ID NO: 37 - DNA, 57 bp, Artificial Sequence
  Description of Artificial Sequence: Synthetic oligonucleotide
gcgcttctcttgcaacacgcactccatgtggtagagtgcgtgttgcaagagaagcgc

SEQ ID NO: 38 - DNA, 57 bp, Artificial Sequence
  Description of Artificial Sequence: Synthetic oligonucleotide
gcgctcaggactaggtgcagactccatgtggtagagtctgcacctagtcctgagcgc

SEQ ID NO: 39 - DNA, 57 bp, Artificial Sequence
  Description of Artificial Sequence: Synthetic oligonucleotide
gcgcgatcgagtgttgaataactccatgtggtagagttattcaacactcgatcgcgc

SEQ ID NO: 40 - DNA, 57 bp, Artificial Sequence
  Description of Artificial Sequence: Synthetic oligonucleotide
gcgccagtaccctggagaaacctccatgtggtagaggtttctccagggtactggcgc

SEQ ID NO: 41 - DNA, 57 bp, Artificial Sequence
  Description of Artificial Sequence: Synthetic oligonucleotide
gcgccactgtccacaggagaactccatgtggtagagttctcctgtggacagtggcgc

SEQ ID NO: 42 - DNA, 57 bp, Artificial Sequence
  Description of Artificial Sequence: Synthetic oligonucleotide
gcgcacagtaccctggagaaactccatgtggtagagtttctccagggtactgtgcgc

SEQ ID NO: 43 - DNA, 64 bp, Artificial Sequence; identical to SEQ ID NO: 1
  Description of Artificial Sequence: Synthetic oligonucleotide

SEQ ID NO: 44 - DNA, 64 bp, Artificial Sequence; identical to SEQ ID NO: 2
  Description of Artificial Sequence: Synthetic oligonucleotide

SEQ ID NO: 45 - DNA, 57 bp, Artificial Sequence
  Description of Artificial Sequence: Synthetic oligonucleotide
caacaagatgaagagcaccaactccatgtggtagagttggtgctcttcatcttgttg

SEQ ID NO: 46 - DNA, 21 bp, Artificial Sequence
  Description of Artificial Sequence: Synthetic oligonucleotide
cgcacagaacactcatggatt

SEQ ID NO: 47 - DNA, 21 bp, Artificial Sequence
  Description of Artificial Sequence: Synthetic oligonucleotide
ccagaggatgacgattgttta

SEQ ID NO: 48 - DNA, 21 bp, Artificial Sequence
  Description of Artificial Sequence: Synthetic oligonucleotide
tcggagactccagacaatcgc

SEQ ID NO: 49 - DNA, 21 bp, Artificial Sequence
  Description of Artificial Sequence: Synthetic oligonucleotide
cctccaggcagctcaaagatc

SEQ ID NO: 50 - DNA, 21 bp, Artificial Sequence
  Description of Artificial Sequence: Synthetic oligonucleotide
tcaggactaggtgcagaatgt

SEQ ID NO: 51 - DNA, 21 bp, Artificial Sequence
  Description of Artificial Sequence: Synthetic oligonucleotide
ttctcttgcaacacgcacaga

SEQ ID NO: 52 - DNA, 21 bp, Artificial Sequence
  Description of Artificial Sequence: Synthetic oligonucleotide
gatcgagtgttgaataatgat

SEQ ID NO: 53 - DNA, 21 bp, Artificial Sequence
  Description of Artificial Sequence: Synthetic oligonucleotide
cagtaccctggagaaacacat

SEQ ID NO: 54 - DNA, 21 bp, Artificial Sequence
  Description of Artificial Sequence: Synthetic oligonucleotide
cactgtccacaggagaagcca

SEQ ID NO: 55 - DNA, 21 bp, Artificial Sequence
  Description of Artificial Sequence: Synthetic oligonucleotide
acagtaccctggagaaacaca

SEQ ID NO: 56 - DNA, 21 bp, Artificial Sequence
  Description of Artificial Sequence: Synthetic oligonucleotide
caacaagatgaagagcaccaa

SEQ ID NO: 57 - DNA, 21 bp, Artificial Sequence
  Description of Artificial Sequence: Synthetic oligonucleotide
gcgccgcacagaacactcatg

SEQ ID NO: 58 - DNA, 21 bp, Artificial Sequence
  Description of Artificial Sequence: Synthetic oligonucleotide
gcgctcggagactccagacaa

SEQ ID NO: 59 - DNA, 21 bp, Artificial Sequence
  Description of Artificial Sequence: Synthetic oligonucleotide
gcgccctccaggcagctcaaa

SEQ ID NO: 60 - DNA, 21 bp, Artificial Sequence
  Description of Artificial Sequence: Synthetic oligonucleotide
gcgctcaggactaggtgcaga

SEQ ID NO: 61 - DNA, 21 bp, Artificial Sequence
  Description of Artificial Sequence: Synthetic oligonucleotide
gcgcgatcgagtgttgaataa

SEQ ID NO: 62 - DNA, 21 bp, Artificial Sequence
  Description of Artificial Sequence: Synthetic oligonucleotide
gcgccagtaccctggagaaac

SEQ ID NO: 63 - DNA, 21 bp, Artificial Sequence
  Description of Artificial Sequence: Synthetic oligonucleotide
gcgccactgtccacaggagaa

SEQ ID NO: 64 - DNA, 21 bp, Artificial Sequence
  Description of Artificial Sequence: Synthetic oligonucleotide
gcgcttctcttgcaacacgca

SEQ ID NO: 65 - DNA, 21 bp, Artificial Sequence
  Description of Artificial Sequence: Synthetic oligonucleotide
gcgcacagtaccctggagaaa

SEQ ID NO: 66 - DNA, 21 bp, Artificial Sequence
  Description of Artificial Sequence: Synthetic oligonucleotide
cgcacagaacactcatggatt

SEQ ID NO: 67 - DNA, 26 bp, Artificial Sequence
  Description of Artificial Sequence: Synthetic oligonucleotide
acgctcgcacagaacactcatggatt

SEQ ID NO: 68 - DNA, 15 bp, Artificial Sequence
  Description of Artificial Sequence: Synthetic oligonucleotide
ctccatgtggtagag

SEQ ID NO: 69 - DNA, 21 bp, Artificial Sequence
  Description of Artificial Sequence: Synthetic primer
gaagcagaggacaagttccca

SEQ ID NO: 70 - DNA, 19 bp, Artificial Sequence
  Description of Artificial Sequence: Synthetic primer
tcaccaccatggagaaggc

SEQ ID NO: 71 - DNA, 20 bp, Artificial Sequence
  Description of Artificial Sequence: Synthetic primer
gctaagcagttggtggtgca

SEQ ID NO: 72 - DNA, 19 bp, Artificial Sequence
  Description of Artificial Sequence: Synthetic primer
tggatgatctcaagggcac

SEQ ID NO: 73 - DNA, 20 bp, Artificial Sequence
  Description of Artificial Sequence: Synthetic primer
tcagtggtatctggaggaca

SEQ ID NO: 74 - DNA, 21 bp, Artificial Sequence
  Description of Artificial Sequence: Synthetic primer
ctgaggagaagtctgccgtta

SEQ ID NO: 75 - DNA, 20 bp, Artificial Sequence
  Description of Artificial Sequence: Synthetic primer
agcatcaggagtggacagat

SEQ ID NO: 76 - DNA, 20 bp, Artificial Sequence
  Description of Artificial Sequence: Synthetic primer
acccagaagactgtggatgg

SEQ ID NO: 77 - DNA, 20 bp, Artificial Sequence
  Description of Artificial Sequence: Synthetic primer
ttcagctcagggatgacctt

SEQ ID NO: 78 - DNA, 20 bp, Artificial Sequence
  Description of Artificial Sequence: Synthetic probe
cggagactccagacaatcgc

SEQ ID NO: 79 - DNA, 20 bp, Artificial Sequence
  Description of Artificial Sequence: Synthetic probe
ctccaggcagctcaaagatc

SEQ ID NO: 80 - DNA, 20 bp, Artificial Sequence
  Description of Artificial Sequence: Synthetic probe
tctcttgcaacacgcacaga

SEQ ID NO: 81 - DNA, 20 bp, Artificial Sequence
  Description of Artificial Sequence: Synthetic probe
caggactaggtgcagaatgt

SEQ ID NO: 82 - DNA, 20 bp, Artificial Sequence
  Description of Artificial Sequence: Synthetic probe
atcgagtgttgaataatgat

SEQ ID NO: 83 - DNA, 19 bp, Artificial Sequence
  Description of Artificial Sequence: Synthetic probe
gtaccctggagaaacacat

SEQ ID NO: 84 - DNA, 20 bp, Artificial Sequence
  Description of Artificial Sequence: Synthetic probe
actgtccacaggagaagcca

SEQ ID NO: 85 - DNA, 20 bp, Artificial Sequence
  Description of Artificial Sequence: Synthetic probe
cagtaccctggagaaacaca

SEQ ID NO: 86 - DNA, 57 bp, Artificial Sequence
  Description of Artificial Sequence: Synthetic oligonucleotide
ccggcgcacagaacactcatggattctcgagaatccatgagtgttctgtgcgttttt

SEQ ID NO: 87 - DNA, 65 bp, Artificial Sequence
  Description of Artificial Sequence: Synthetic oligonucleotide
cgctcgcacagaacactcatggattctccatgtggtagagaatccatgagtgttctgtgcgagtg

SEQ ID NO: 88 - DNA, 65 bp, Artificial Sequence
  Description of Artificial Sequence: Synthetic oligonucleotide
cgctgcgccgcacagaacactcatgctccatgtggtagagcatgagtgttctgtgcggcgcagtg

SEQ ID NO: 89 - DNA, 57 bp, Artificial Sequence
  Description of Artificial Sequence: Synthetic oligonucleotide
ccggacagtaccctggagaaacacactcgagtgtgtttctccagggtactgtttttt

SEQ ID NO: 90 - DNA, 65 bp, Artificial Sequence
  Description of Artificial Sequence: Synthetic oligonucleotide
cgctacagtaccctggagaaacacactccatgtggtagagtgtgtttctccagggtactgtagtg

SEQ ID NO: 91 - DNA, 65 bp, Artificial Sequence
  Description of Artificial Sequence: Synthetic oligonucleotide
cgctgcgcacagtaccctggagaaactccatgtggtagagtttctccagggtactgtgcgcagtg

SEQ ID NO: 92 - DNA, 57 bp, Artificial Sequence
  Description of Artificial Sequence: Synthetic oligonucleotide
ccggttctcttgcaacacgcacagactcgagtctgtgcgtgttgcaagagaattttt

SEQ ID NO: 93 - DNA, 65 bp, Artificial Sequence
  Description of Artificial Sequence: Synthetic oligonucleotide
cgctttctcttgcaacacgcacagactccatgtggtagagtctgtgcgtgttgcaagagaaagtg

SEQ ID NO: 94 - DNA, 65 bp, Artificial Sequence
  Description of Artificial Sequence: Synthetic oligonucleotide
cgctgcgcttctcttgcaacacgcactccatgtggtagagtgcgtgttgcaagagaagcgcagtg

SEQ ID NO: 95 - DNA, 57 bp, Artificial Sequence
  Description of Artificial Sequence: Synthetic oligonucleotide
ccgggatcgagtgttgaataatgatctcgagatcattattcaacactcgatcttttt

SEQ ID NO: 96 - DNA, 65 bp, Artificial Sequence
  Description of Artificial Sequence: Synthetic oligonucleotide
cgctgatcgagtgttgaataatgatctccatgtggtagagatcattattcaacactcgatcagtg

SEQ ID NO: 97 - DNA, 65 bp, Artificial Sequence
  Description of Artificial Sequence: Synthetic oligonucleotide
cgctgcgcgatcgagtgttgaataactccatgtggtagagttattcaacactcgatcgcgcagtg

SEQ ID NO: 98 - DNA, 21 bp, Artificial Sequence
  Description of Artificial Sequence: Synthetic primer
tggcctgtggagtaaggtcaa

SEQ ID NO: 99 - DNA, 52 bp, Artificial Sequence
  Description of Artificial Sequence: Synthetic oligonucleotide
  modified_base (1)..(21): a, c, t, g, unknown or other
  modified_base (28)..(47): a, c, t, g, unknown or other
nnnnnnnnnnnnnnnnnnnnnctcgagnnnnnnnnnnnnnnnnnnnnttttt

SEQ ID NO: 100 - DNA, 51 bp, Artificial Sequence
  Description of Artificial Sequence: Synthetic oligonucleotide
  modified_base (5)..(24): a, c, t, g, unknown or other
  modified_base (31)..(51): a, c, t, g, unknown or other
aaaannnnnnnnnnnnnnnnnnnnctcgagnnnnnnnnnnnnnnnnnnnnn

SEQ ID NO: 101 - DNA, 64 bp, Artificial Sequence
  Description of Artificial Sequence: Synthetic oligonucleotide
  modified_base (5)..(25): a, c, t, g, unknown or other
  modified_base (41)..(60): a, c, t, g, unknown or other
ccggnnnnnnnnnnnnnnnnnnnnnctccatgtggtagagnnnnnnnnnnnnnnnnnnnncggc

SEQ ID NO: 102 - DNA, 64 bp, Artificial Sequence
  Description of Artificial Sequence: Synthetic oligonucleotide
  modified_base (5)..(24): a, c, t, g, unknown or other
  modified_base (40)..(60): a, c, t, g, unknown or other
gccgnnnnnnnnnnnnnnnnnnnnctctaccacatggagnnnnnnnnnnnnnnnnnnnnnccgg

SEQ ID NO: 103 - DNA, 58 bp, Artificial Sequence
  Description of Artificial Sequence: Synthetic oligonucleotide
  modified_base (5)..(25): a, c, t, g, unknown or other
  modified_base (32)..(52): a, c, t, g, unknown or other
ccggnnnnnnnnnnnnnnnnnnnnnctcgagnnnnnnnnnnnnnnnnnnnnntttttg

SEQ ID NO: 104 - DNA, 39 bp, Artificial Sequence
  Description of Artificial Sequence: Synthetic oligonucleotide
  modified_base (5)..(15): a, c, t, g, unknown or other
  modified_base (23)..(33): a, c, t, g, unknown or other
gcccnnnnnnnnnnntcttgaannnnnnnnnnngggcct

SEQ ID NO: 105 - DNA, 31 bp, Artificial Sequence
  Description of Artificial Sequence: Synthetic oligonucleotide
tagagaatccatgagtgttctgtgcgagtgc

SEQ ID NO: 106 - DNA, 22 bp, Artificial Sequence
  Description of Artificial Sequence: Synthetic oligonucleotide
aatccatgagtgttctgtgcga

SEQ ID NO: 107 - DNA, 21 bp, Artificial Sequence
  Description of Artificial Sequence: Synthetic oligonucleotide
aatccatgagtgttctgtgcg

SEQ ID NO: 108 - DNA, 21 bp, Artificial Sequence
  Description of Artificial Sequence: Synthetic oligonucleotide
atccatgagtgttctgtgcga

SEQ ID NO: 109 - DNA, 20 bp, Artificial Sequence
  Description of Artificial Sequence: Synthetic oligonucleotide
aatccatgagtgttctgtgc

SEQ ID NO: 110 - DNA, 22 bp, Artificial Sequence
  Description of Artificial Sequence: Synthetic oligonucleotide
aatccatgagtgttctgtgcgg

SEQ ID NO: 111 - DNA, 23 bp, Artificial Sequence
  Description of Artificial Sequence: Synthetic oligonucleotide
gaatccatgagtgttctgtgcga

SEQ ID NO: 112 - DNA, 22 bp, Artificial Sequence
  Description of Artificial Sequence: Synthetic oligonucleotide
aatccatgagtgttctgtgcgt

SEQ ID NO: 113 - DNA, 22 bp, Artificial Sequence
  Description of Artificial Sequence: Synthetic oligonucleotide
aatccatgagtgttctgtgcgc

SEQ ID NO: 114 - DNA, 22 bp, Artificial Sequence
  Description of Artificial Sequence: Synthetic oligonucleotide
gaatccatgagtgttctgtgcg

SEQ ID NO: 115 - DNA, 21 bp, Artificial Sequence
  Description of Artificial Sequence: Synthetic oligonucleotide
aatccatgagtgttctgtgca

SEQ ID NO: 116 - DNA, 33 bp, Artificial Sequence
  Description of Artificial Sequence: Synthetic oligonucleotide
ctcgagaatccatgagtgttctgtgcgtttttg

SEQ ID NO: 117 - DNA, 21 bp, Artificial Sequence
  Description of Artificial Sequence: Synthetic oligonucleotide
catgagtgttctgtgcgtttt

SEQ ID NO: 118 - DNA, 22 bp, Artificial Sequence
  Description of Artificial Sequence: Synthetic oligonucleotide
catgagtgttctgtgcgttttt

SEQ ID NO: 119 - DNA, 20 bp, Artificial Sequence
  Description of Artificial Sequence: Synthetic oligonucleotide
catgagtgttctgtgcgttt

SEQ ID NO: 120 - DNA, 23 bp, Artificial Sequence
  Description of Artificial Sequence: Synthetic oligonucleotide
tccatgagtgttctgtgcgtttt

SEQ ID NO: 121 - DNA, 21 bp, Artificial Sequence
  Description of Artificial Sequence: Synthetic oligonucleotide
catgagtgttctgtgcgttta

SEQ ID NO: 122 - DNA, 21 bp, Artificial Sequence
  Description of Artificial Sequence: Synthetic oligonucleotide
catgagtgttctgtgcgtttc

SEQ ID NO: 123 - DNA, 22 bp, Artificial Sequence
  Description of Artificial Sequence: Synthetic oligonucleotide
catgagtgttctgtgcgtttat

SEQ ID NO: 124 - DNA, 22 bp, Artificial Sequence
  Description of Artificial Sequence: Synthetic oligonucleotide
tccatgagtgttctgtgcgttt

SEQ ID NO: 125 - DNA, 19 bp, Artificial Sequence
  Description of Artificial Sequence: Synthetic oligonucleotide
catgagtgttctgtgcgtt

SEQ ID NO: 126 - DNA, 23 bp, Artificial Sequence
  Description of Artificial Sequence: Synthetic oligonucleotide
catgagtgttctgtgcgtttttt

SEQ ID NO: 127 - DNA, 31 bp, Artificial Sequence
  Description of Artificial Sequence: Synthetic oligonucleotide
tagagtgtgtttctccagggtactgtagtgc

SEQ ID NO: 128 - DNA, 19 bp, Artificial Sequence
  Description of Artificial Sequence: Synthetic oligonucleotide
tgtttctccagggtactgt

SEQ ID NO: 129 - DNA, 17 bp, Artificial Sequence
  Description of Artificial Sequence: Synthetic oligonucleotide
tttctccagggtactgt

SEQ ID NO: 130 - DNA, 18 bp, Artificial Sequence
  Description of Artificial Sequence: Synthetic oligonucleotide
tgtttctccagggtactg

SEQ ID NO: 131 - DNA, 21 bp, Artificial Sequence
  Description of Artificial Sequence: Synthetic oligonucleotide
tgtgtttctccagggtactgt

SEQ ID NO: 132 - DNA, 16 bp, Artificial Sequence
  Description of Artificial Sequence: Synthetic oligonucleotide
tttctccagggtactg

SEQ ID NO: 133 - DNA, 17 bp, Artificial Sequence
  Description of Artificial Sequence: Synthetic oligonucleotide
tgtttctccagggtact

SEQ ID NO: 134 - DNA, 20 bp, Artificial Sequence
  Description of Artificial Sequence: Synthetic oligonucleotide
tgtgtttctccagggtactg

SEQ ID NO: 135 - DNA, 33 bp, Artificial Sequence
  Description of Artificial Sequence: Synthetic oligonucleotide
ctcgagtgtgtttctccagggtactgttttttg

SEQ ID NO: 136 - DNA, 18 bp, Artificial Sequence
  Description of Artificial Sequence: Synthetic oligonucleotide
tttctccagggtactgtt

SEQ ID NO: 137 - DNA, 20 bp, Artificial Sequence
  Description of Artificial Sequence: Synthetic oligonucleotide
tgtttctccagggtactgtt

SEQ ID NO: 138 - DNA, 21 bp, Artificial Sequence
  Description of Artificial Sequence: Synthetic oligonucleotide
tttctccagggtactgttttt

SEQ ID NO: 139 - DNA, 20 bp, Artificial Sequence
  Description of Artificial Sequence: Synthetic oligonucleotide
tttctccagggtactgtttt

SEQ ID NO: 140 - DNA, 19 bp, Artificial Sequence
  Description of Artificial Sequence: Synthetic oligonucleotide
tttctccagggtactgttt

SEQ ID NO: 141 - DNA, 71 bp, Artificial Sequence
  Description of Artificial Sequence: Synthetic oligonucleotide
  modified_base (9)..(29): a, c, t, g, unknown or other
  modified_base (45)..(65): a, c, t, g, unknown or other
gccacgctnnnnnnnnnnnnnnnnnnnnnctccatgtggtagagnnnnnnnnnnnnnnnnnnnnnagtgcg

SEQ ID NO: 142 - DNA, 31 bp, Artificial Sequence
  Description of Artificial Sequence: Synthetic oligonucleotide
tagagcatgagtgttctgtgcggcgcagtgc

SEQ ID NO: 143 - DNA, 21 bp, Artificial Sequence
  Description of Artificial Sequence: Synthetic oligonucleotide
catgagtgttctgtgcggcgc

SEQ ID NO: 144 - DNA, 20 bp, Artificial Sequence
  Description of Artificial Sequence: Synthetic oligonucleotide
catgagtgttctgtgcggcg

SEQ ID NO: 145 - DNA, 19 bp, Artificial Sequence
  Description of Artificial Sequence: Synthetic oligonucleotide
catgagtgttctgtgcggc

SEQ ID NO: 146 - DNA, 20 bp, Artificial Sequence
  Description of Artificial Sequence: Synthetic oligonucleotide
atgagtgttctgtgcggcgc

SEQ ID NO: 147 - DNA, 18 bp, Artificial Sequence
  Description of Artificial Sequence: Synthetic oligonucleotide
catgagtgttctgtgcgg

SEQ ID NO: 148 - DNA, 19 bp, Artificial Sequence
  Description of Artificial Sequence: Synthetic oligonucleotide
atgagtgttctgtgcggcg

SEQ ID NO: 149 - DNA, 16 bp, Artificial Sequence
  Description of Artificial Sequence: Synthetic oligonucleotide
catgagtgttctgtgc

SEQ ID NO: 150 - DNA, 19 bp, Artificial Sequence
  Description of Artificial Sequence: Synthetic oligonucleotide
tgagtgttctgtgcggcgc

SEQ ID NO: 151 - DNA, 31 bp, Artificial Sequence
  Description of Artificial Sequence: Synthetic oligonucleotide
tagagtttctccagggtactgtgcgcagtgc

SEQ ID NO: 152 - DNA, 20 bp, Artificial Sequence
  Description of Artificial Sequence: Synthetic oligonucleotide
tttctccagggtactgtgcg

SEQ ID NO: 153 - DNA, 19 bp, Artificial Sequence
  Description of Artificial Sequence: Synthetic oligonucleotide
tttctccagggtactgtgc

SEQ ID NO: 154 - DNA, 21 bp, Artificial Sequence
  Description of Artificial Sequence: Synthetic oligonucleotide
gtttctccagggtactgtgcg

SEQ ID NO: 155 - DNA, 21 bp, Artificial Sequence
  Description of Artificial Sequence: Synthetic oligonucleotide
tttctccagggtactgtgcgc

SEQ ID NO: 156 - DNA, 18 bp, Artificial Sequence
  Description of Artificial Sequence: Synthetic oligonucleotide
tttctccagggtactgtg

SEQ ID NO: 157 - DNA, 20 bp, Artificial Sequence
  Description of Artificial Sequence: Synthetic oligonucleotide
gtttctccagggtactgtgc

SEQ ID NO: 158 - DNA, 32 bp, Artificial Sequence
  Description of Artificial Sequence: Synthetic oligonucleotide
ctcgagaatccatgagtgttctgtgcgttttt

SEQ ID NO: 159 - DNA, 33 bp, Artificial Sequence
  Description of Artificial Sequence: Synthetic oligonucleotide
ctcgagtctgtgcgtgttgcaagagaatttttg

SEQ ID NO: 160 - DNA, 23 bp, Artificial Sequence
  Description of Artificial Sequence: Synthetic oligonucleotide
tgtgcgtgttgcaagagaatttt

SEQ ID NO: 161 - DNA, 22 bp, Artificial Sequence
  Description of Artificial Sequence: Synthetic oligonucleotide
tgtgcgtgttgcaagagaattt

SEQ ID NO: 162 - DNA, 21 bp, Artificial Sequence
  Description of Artificial Sequence: Synthetic oligonucleotide
tgtgcgtgttgcaagagaatt

SEQ ID NO: 163 - DNA, 24 bp, Artificial Sequence
  Description of Artificial Sequence: Synthetic oligonucleotide
tgtgcgtgttgcaagagaattttg

SEQ ID NO: 164 - DNA, 23 bp, Artificial Sequence
  Description of Artificial Sequence: Synthetic oligonucleotide
  modified_base (5)..(5): a, c, t, g, unknown or other
tgtgngtgttgcaagagaatttt

SEQ ID NO: 165 - DNA, 20 bp, Artificial Sequence
  Description of Artificial Sequence: Synthetic oligonucleotide
tgtgcgtgttgcaagagaat

SEQ ID NO: 166 - DNA, 24 bp, Artificial Sequence
  Description of Artificial Sequence: Synthetic oligonucleotide
tgtgcgtgttgcaagagaattttt

SEQ ID NO: 167 - DNA, 22 bp, Artificial Sequence
  Description of Artificial Sequence: Synthetic oligonucleotide
  modified_base (5)..(5): a, c, t, g, unknown or other
tgtgngtgttgcaagagaattt

SEQ ID NO: 168 - DNA, 21 bp, Artificial Sequence
  Description of Artificial Sequence: Synthetic oligonucleotide
  modified_base (5)..(5): a, c, t, g, unknown or other
tgtgngtgttgcaagagaatt

SEQ ID NO: 169 - DNA, 24 bp, Artificial Sequence
  Description of Artificial Sequence: Synthetic oligonucleotide
tgtgcgtgttgcaagagaatttta

SEQ ID NO: 170 - DNA, 31 bp, Artificial Sequence
  Description of Artificial Sequence: Synthetic oligonucleotide
ctcgaggcgattgtctggagtctccgatttt

SEQ ID NO: 171 - DNA, 17 bp, Artificial Sequence
  Description of Artificial Sequence: Synthetic oligonucleotide
attgtctggagtctccg

SEQ ID NO: 172 - DNA, 18 bp, Artificial Sequence
  Description of Artificial Sequence: Synthetic oligonucleotide
attgtctggagtctccga

SEQ ID NO: 173 - DNA, 16 bp, Artificial Sequence
  Description of Artificial Sequence: Synthetic oligonucleotide
attgtctggagtctcc

SEQ ID NO: 174 - DNA, 19 bp, Artificial Sequence
  Description of Artificial Sequence: Synthetic oligonucleotide
gattgtctggagtctccga

SEQ ID NO: 175 - DNA, 16 bp, Artificial Sequence
  Description of Artificial Sequence: Synthetic oligonucleotide
ttgtctggagtctccg

SEQ ID NO: 176 - DNA, 20 bp, Artificial Sequence
  Description of Artificial Sequence: Synthetic oligonucleotide
attgtctggagtctccgatt

SEQ ID NO: 177 - DNA, 17 bp, Artificial Sequence
  Description of Artificial Sequence: Synthetic oligonucleotide
ttgtctggagtctccga

SEQ ID NO: 178 - DNA, 18 bp, Artificial Sequence
  Description of Artificial Sequence: Synthetic oligonucleotide
gattgtctggagtctccg

SEQ ID NO: 179 - DNA, 21 bp, Artificial Sequence
  Description of Artificial Sequence: Synthetic oligonucleotide
gattgtctggagtctccgatt

SEQ ID NO: 180 - DNA, 19 bp, Artificial Sequence
  Description of Artificial Sequence: Synthetic oligonucleotide
attgtctggagtctccgat

SEQ ID NO: 181 - DNA, 32 bp, Artificial Sequence
  Description of Artificial Sequence: Synthetic oligonucleotide
ctcgagacattctgcacctagtcctgattttt

SEQ ID NO: 182 - DNA, 20 bp, Artificial Sequence
  Description of Artificial Sequence: Synthetic oligonucleotide
ttctgcacctagtcctgatt

SEQ ID NO: 183 - DNA, 22 bp, Artificial Sequence
  Description of Artificial Sequence: Synthetic oligonucleotide
ttctgcacctagtcctgatttt

SEQ ID NO: 184 - DNA, 19 bp, Artificial Sequence
  Description of Artificial Sequence: Synthetic oligonucleotide
ttctgcacctagtcctgat

SEQ ID NO: 185 - DNA, 21 bp, Artificial Sequence
  Description of Artificial Sequence: Synthetic oligonucleotide
ttctgcacctagtcctgattt

SEQ ID NO: 186 - DNA, 21 bp, Artificial Sequence
  Description of Artificial Sequence: Synthetic oligonucleotide
attctgcacctagtcctgatt

SEQ ID NO: 187 - DNA, 20 bp, Artificial Sequence
  Description of Artificial Sequence: Synthetic oligonucleotide
ttctgcacctagtcctgatc

SEQ ID NO: 188 - DNA, 20 bp, Artificial Sequence
  Description of Artificial Sequence: Synthetic oligonucleotide
ttctgcacctagtcctgata

SEQ ID NO: 189 - DNA, 23 bp, Artificial Sequence
  Description of Artificial Sequence: Synthetic oligonucleotide
ttctgcacctagtcctgattttt

SEQ ID NO: 190 - DNA, 23 bp, Artificial Sequence
  Description of Artificial Sequence: Synthetic oligonucleotide
attctgcacctagtcctgatttt

SEQ ID NO: 191 - DNA, 18 bp, Artificial Sequence
  Description of Artificial Sequence: Synthetic oligonucleotide
ttctgcacctagtcctga

SEQ ID NO: 192 - DNA, 32 bp, Artificial Sequence
  Description of Artificial Sequence: Synthetic oligonucleotide
ctcgagtgtgtttctccagggtactgtttttt

SEQ ID NO: 193 - DNA, 22 bp, Artificial Sequence
  Description of Artificial Sequence: Synthetic oligonucleotide
tttctccagggtactgtttttt

SEQ ID NO: 194 - DNA, 32 bp, Artificial Sequence
  Description of Artificial Sequence: Synthetic oligonucleotide
ctcgagatgtgtttctccagggtactgttttt

SEQ ID NO: 195 - DNA, 22 bp, Artificial Sequence
  Description of Artificial Sequence: Synthetic oligonucleotide
tgtttctccagggtactgtttt

SEQ ID NO: 196 - DNA, 21 bp, Artificial Sequence
  Description of Artificial Sequence: Synthetic oligonucleotide
tgtttctccagggtactgttt

SEQ ID NO: 197 - DNA, 23 bp, Artificial Sequence
  Description of Artificial Sequence: Synthetic oligonucleotide
tgtttctccagggtactgttttt

SEQ ID NO: 198 - DNA, 20 bp, Artificial Sequence
  Description of Artificial Sequence: Synthetic oligonucleotide
tgtttctccagggtactgta

SEQ ID NO: 199 - DNA, 21 bp, Artificial Sequence
  Description of Artificial Sequence: Synthetic oligonucleotide
tgtttctccagggtactgtta

SEQ ID NO: 200 - DNA, 32 bp, Artificial Sequence
  Description of Artificial Sequence: Synthetic oligonucleotide
ctcgaggatctttgagctgcctggaggttttt

SEQ ID NO: 201 - DNA, 19 bp, Artificial Sequence
  Description of Artificial Sequence: Synthetic oligonucleotide
tttgagctgcctggaggtt

SEQ ID NO: 202 - DNA, 21 bp, Artificial Sequence
  Description of Artificial Sequence: Synthetic oligonucleotide
tttgagctgcctggaggttta

SEQ ID NO: 203 - DNA, 21 bp, Artificial Sequence
  Description of Artificial Sequence: Synthetic oligonucleotide
tttgagctgcctggaggtttc

SEQ ID NO: 204 - DNA, 20 bp, Artificial Sequence
  Description of Artificial Sequence: Synthetic oligonucleotide
tttgagctgcctggaggttc

SEQ ID NO: 205 - DNA, 23 bp, Artificial Sequence
  Description of Artificial Sequence: Synthetic oligonucleotide
tttgagctgcctggaggtttttt

SEQ ID NO: 206 - DNA, 24 bp, Artificial Sequence
  Description of Artificial Sequence: Synthetic oligonucleotide
tctttgagctgcctggaggttttt

SEQ ID NO: 207 - DNA, 18 bp, Artificial Sequence
  Description of Artificial Sequence: Synthetic oligonucleotide
tttgagctgcctggaggt

SEQ ID NO: 208 - DNA, 20 bp, Artificial Sequence
  Description of Artificial Sequence: Synthetic oligonucleotide
tttgagctgcctggaggtta

SEQ ID NO: 209 - DNA, 22 bp, Artificial Sequence
  Description of Artificial Sequence: Synthetic oligonucleotide
tttgagctgcctggaggtttat

SEQ ID NO: 210 - DNA, 22 bp, Artificial Sequence
  Description of Artificial Sequence: Synthetic oligonucleotide
tttgagctgcctggaggttttg

SEQ ID NO: 211 - DNA, 32 bp, Artificial Sequence
  Description of Artificial Sequence: Synthetic oligonucleotide
tagagtctgtgcgtgttgcaagagaaagtgcg

SEQ ID NO: 212 - DNA, 20 bp, Artificial Sequence
  Description of Artificial Sequence: Synthetic oligonucleotide
tctgtgcgtgttgcaagaga

SEQ ID NO: 213 - DNA, 22 bp, Artificial Sequence
  Description of Artificial Sequence: Synthetic oligonucleotide
tctgtgcgtgttgcaagagaaa

SEQ ID NO: 214 - DNA, 21 bp, Artificial Sequence
  Description of Artificial Sequence: Synthetic oligonucleotide
tctgtgcgtgttgcaagagaa

SEQ ID NO: 215 - DNA, 17 bp, Artificial Sequence
  Description of Artificial Sequence: Synthetic oligonucleotide
tctgtgcgtgttgcaag

SEQ ID NO: 216 - DNA, 19 bp, Artificial Sequence
  Description of Artificial Sequence: Synthetic oligonucleotide
tctgtgcgtgttgcaagag

SEQ ID NO: 217 - DNA, 18 bp, Artificial Sequence
  Description of Artificial Sequence: Synthetic oligonucleotide
tctgtgcgtgttgcaaga

SEQ ID NO: 218 - DNA, 19 bp, Artificial Sequence
  Description of Artificial Sequence: Synthetic oligonucleotide
ctgtgcgtgttgcaagaga

SEQ ID NO: 219 - DNA, 21 bp, Artificial Sequence
  Description of Artificial Sequence: Synthetic oligonucleotide
ctgtgcgtgttgcaagagaaa

SEQ ID NO: 220 - DNA, 20 bp, Artificial Sequence
  Description of Artificial Sequence: Synthetic oligonucleotide
ctgtgcgtgttgcaagagaa

SEQ ID NO: 221 - DNA, 16 bp, Artificial Sequence
  Description of Artificial Sequence: Synthetic oligonucleotide
tctgtgcgtgttgcaa

SEQ ID NO: 222 - DNA, 31 bp, Artificial Sequence
  Description of Artificial Sequence: Synthetic oligonucleotide
tagaggcgattgtctggagtctccgaagtgc

SEQ ID NO: 223 - DNA, 21 bp, Artificial Sequence
  Description of Artificial Sequence: Synthetic oligonucleotide
gcgattgtctggagtctccga

SEQ ID NO: 224 - DNA, 20 bp, Artificial Sequence
  Description of Artificial Sequence: Synthetic oligonucleotide
cgattgtctggagtctccga

SEQ ID NO: 225 - DNA, 22 bp, Artificial Sequence
  Description of Artificial Sequence: Synthetic oligonucleotide
gcgattgtctggagtctccgaa

SEQ ID NO: 226 - DNA, 22 bp, Artificial Sequence
  Description of Artificial Sequence: Synthetic oligonucleotide
ggcgattgtctggagtctccga

SEQ ID NO: 227 - DNA, 21 bp, Artificial Sequence
  Description of Artificial Sequence: Synthetic oligonucleotide
cgattgtctggagtctccgaa

SEQ ID NO: 228 - DNA, 19 bp, Artificial Sequence
  Description of Artificial Sequence: Synthetic oligonucleotide
cgattgtctggagtctccg

SEQ ID NO: 229 - DNA, 20 bp, Artificial Sequence
  Description of Artificial Sequence: Synthetic oligonucleotide
gcgattgtctggagtctccg

SEQ ID NO: 230 - DNA, 23 bp, Artificial Sequence
  Description of Artificial Sequence: Synthetic oligonucleotide
cgattgtctggagtctccgaatt

SEQ ID NO: 231 - DNA, 23 bp, Artificial Sequence
  Description of Artificial Sequence: Synthetic oligonucleotide
ggcgattgtctggagtctccgaa

SEQ ID NO: 232 - DNA, 23 bp, Artificial Sequence
  Description of Artificial Sequence: Synthetic oligonucleotide
cgattgtctggagtctccgaagt

SEQ ID NO: 233 - DNA, 31 bp, Artificial Sequence
  Description of Artificial Sequence: Synthetic oligonucleotide
tagagacattctgcacctagtcctgaagtgc

SEQ ID NO: 234 - DNA, 21 bp, Artificial Sequence
  Description of Artificial Sequence: Synthetic oligonucleotide
acattctgcacctagtcctga

SEQ ID NO: 235 - DNA, 22 bp, Artificial Sequence
  Description of Artificial Sequence: Synthetic oligonucleotide
acattctgcacctagtcctgaa

SEQ ID NO: 236 - DNA, 23 bp, Artificial Sequence
  Description of Artificial Sequence: Synthetic oligonucleotide
acattctgcacctagtcctgaat

SEQ ID NO: 237 - DNA, 22 bp, Artificial Sequence
  Description of Artificial Sequence: Synthetic oligonucleotide
acattctgcacctagtcctgac

SEQ ID NO: 238 - DNA, 22 bp, Artificial Sequence
  Description of Artificial Sequence: Synthetic oligonucleotide
acattctgcacctagtcctgat

SEQ ID NO: 239 - DNA, 24 bp, Artificial Sequence
  Description of Artificial Sequence: Synthetic oligonucleotide
gacattctgcacctagtcctgaat

SEQ ID NO: 240 - DNA, 20 bp, Artificial Sequence
  Description of Artificial Sequence: Synthetic oligonucleotide
acattctgcacctagtcctg

SEQ ID NO: 241 - DNA, 20 bp, Artificial Sequence
  Description of Artificial Sequence: Synthetic oligonucleotide
cattctgcacctagtcctga

SEQ ID NO: 242 - DNA, 23 bp, Artificial Sequence
  Description of Artificial Sequence: Synthetic oligonucleotide
acattctgcacctagtcctgaaa

SEQ ID NO: 243 - DNA, 23 bp, Artificial Sequence
  Description of Artificial Sequence: Synthetic oligonucleotide
acattctgcacctagtcctgaac

SEQ ID NO: 244 - DNA, 18 bp, Artificial Sequence
  Description of Artificial Sequence: Synthetic oligonucleotide
gtttctccagggtactgt

SEQ ID NO: 245 - DNA, 19 bp, Artificial Sequence
  Description of Artificial Sequence: Synthetic oligonucleotide
tgtgtttctccagggtact

SEQ ID NO: 246 - DNA, 16 bp, Artificial Sequence
  Description of Artificial Sequence: Synthetic oligonucleotide
tgtttctccagggtac

SEQ ID NO: 247 - DNA, 31 bp, Artificial Sequence
  Description of Artificial Sequence: Synthetic oligonucleotide
tagagatgtgtttctccagggtactgagtgc

SEQ ID NO: 248 - DNA, 19 bp, Artificial Sequence
  Description of Artificial Sequence: Synthetic oligonucleotide
atgtgtttctccagggtac

SEQ ID NO: 249 - DNA, 23 bp, Artificial Sequence
  Description of Artificial Sequence: Synthetic oligonucleotide
atgtgtttctccagggtactgag

SEQ ID NO: 250 - DNA, 22 bp, Artificial Sequence
  Description of Artificial Sequence: Synthetic oligonucleotide
tgtgtttctccagggtactgag

SEQ ID NO: 251 - DNA, 24 bp, Artificial Sequence
  Description of Artificial Sequence: Synthetic oligonucleotide
atgtgtttctccagggtactgatt

SEQ ID NO: 252 - DNA, 24 bp, Artificial Sequence
  Description of Artificial Sequence: Synthetic oligonucleotide
atgtgtttctccagggtactgaat

SEQ ID NO: 253 - DNA, 20 bp, Artificial Sequence
  Description of Artificial Sequence: Synthetic oligonucleotide
atgtgtttctccagggtact

SEQ ID NO: 254 - DNA, 21 bp, Artificial Sequence
  Description of Artificial Sequence: Synthetic oligonucleotide
tgtgtttctccagggtactga

SEQ ID NO: 255 - DNA, 21 bp, Artificial Sequence
  Description of Artificial Sequence: Synthetic oligonucleotide
atgtgtttctccagggtactg

SEQ ID NO: 256 - DNA, 22 bp, Artificial Sequence
  Description of Artificial Sequence: Synthetic oligonucleotide
atgtgtttctccagggtactga

SEQ ID NO: 257 - DNA, 31 bp, Artificial Sequence
  Description of Artificial Sequence: Synthetic oligonucleotide
tagaggatctttgagctgcctggaggagtgc

SEQ ID NO: 258 - DNA, 22 bp, Artificial Sequence
  Description of Artificial Sequence: Synthetic oligonucleotide
gatctttgagctgcctggagga

SEQ ID NO: 259 - DNA, 21 bp, Artificial Sequence
  Description of Artificial Sequence: Synthetic oligonucleotide
gatctttgagctgcctggagg

SEQ ID NO: 260 - DNA, 23 bp, Artificial Sequence
  Description of Artificial Sequence: Synthetic oligonucleotide
gatctttgagctgcctggaggat

SEQ ID NO: 261 - DNA, 21 bp, Artificial Sequence
  Description of Artificial Sequence: Synthetic oligonucleotide
atctttgagctgcctggagga

SEQ ID NO: 262 - DNA, 22 bp, Artificial Sequence
  Description of Artificial Sequence: Synthetic oligonucleotide
gatctttgagctgcctggaggt

SEQ ID NO: 263 - DNA, 24 bp, Artificial Sequence
  Description of Artificial Sequence: Synthetic oligonucleotide
gatctttgagctgcctggaggatt

SEQ ID NO: 264 - DNA, 24 bp, Artificial Sequence
  Description of Artificial Sequence: Synthetic oligonucleotide
gatctttgagctgcctggaggaat

SEQ ID NO: 265 - DNA, 23 bp, Artificial Sequence
  Description of Artificial Sequence: Synthetic oligonucleotide
gatctttgagctgcctggaggaa

SEQ ID NO: 266 - DNA, 23 bp, Artificial Sequence
  Description of Artificial Sequence: Synthetic oligonucleotide
atctttgagctgcctggaggaat

SEQ ID NO: 267 - DNA, 23 bp, Artificial Sequence
  Description of Artificial Sequence: Synthetic oligonucleotide
gatctttgagctgcctggaggac

SEQ ID NO: 268 - DNA, 17 bp, Artificial Sequence
  Description of Artificial Sequence: Synthetic oligonucleotide
catgagtgttctgtgcg

SEQ ID NO: 269 - DNA, 32 bp, Artificial Sequence
  Description of Artificial Sequence: Synthetic oligonucleotide
tagagtgcgtgttgcaagagaagcgcagtgcg

SEQ ID NO: 270 - DNA, 20 bp, Artificial Sequence
  Description of Artificial Sequence: Synthetic oligonucleotide
tgcgtgttgcaagagaagcg

SEQ ID NO: 271 - DNA, 21 bp, Artificial Sequence
  Description of Artificial Sequence: Synthetic oligonucleotide
tgcgtgttgcaagagaagcgc

SEQ ID NO: 272 - DNA, 19 bp, Artificial Sequence
  Description of Artificial Sequence: Synthetic oligonucleotide
tgcgtgttgcaagagaagc

SEQ ID NO: 273 - DNA, 22 bp, Artificial Sequence
  Description of Artificial Sequence: Synthetic oligonucleotide
tgcgtgttgcaagagaagcgca

SEQ ID NO: 274 - DNA, 18 bp, Artificial Sequence
  Description of Artificial Sequence: Synthetic oligonucleotide
tgcgtgttgcaagagaag

SEQ ID NO: 275 - DNA, 21 bp, Artificial Sequence
  Description of Artificial Sequence: Synthetic oligonucleotide
gtgcgtgttgcaagagaagcg

SEQ ID NO: 276 - DNA, 16 bp, Artificial Sequence
  Description of Artificial Sequence: Synthetic oligonucleotide
tgcgtgttgcaagaga

SEQ ID NO: 277 - DNA, 24 bp, Artificial Sequence
  Description of Artificial Sequence: Synthetic oligonucleotide
tgcgtgttgcaagagaagcgcatt

SEQ ID NO: 278 - DNA, 24 bp, Artificial Sequence
  Description of Artificial Sequence: Synthetic oligonucleotide
tgcgtgttgcaagagaagcgcagt

SEQ ID NO: 279 - DNA, 22 bp, Artificial Sequence
  Description of Artificial Sequence: Synthetic oligonucleotide
gtgcgtgttgcaagagaagcgc

SEQ ID NO: 280 - DNA, 31 bp, Artificial Sequence
  Description of Artificial Sequence: Synthetic oligonucleotide
tagagttgtctggagtctccgagcgcagtgc

SEQ ID NO: 281 - DNA, 16 bp, Artificial Sequence
  Description of Artificial Sequence: Synthetic oligonucleotide
tgtctggagtctccga

SEQ ID NO: 282 - DNA, 20 bp, Artificial Sequence
  Description of Artificial Sequence: Synthetic oligonucleotide
ttgtctggagtctccgagcg

SEQ ID NO: 283 - DNA, 18 bp, Artificial Sequence
  Description of Artificial Sequence: Synthetic oligonucleotide
gttgtctggagtctccga

SEQ ID NO: 284 - DNA, 17 bp, Artificial Sequence
  Description of Artificial Sequence: Synthetic oligonucleotide
gtctggagtctccgagc

SEQ ID NO: 285 - DNA, 16 bp, Artificial Sequence
  Description of Artificial Sequence: Synthetic oligonucleotide
gtctggagtctccgag

SEQ ID NO: 286 - DNA, 31 bp, Artificial Sequence
  Description of Artificial Sequence: Synthetic oligonucleotide
tagagtctgcacctagtcctgagcgcagtgc

SEQ ID NO: 287 - DNA, 21 bp, Artificial Sequence
  Description of Artificial Sequence: Synthetic oligonucleotide
tctgcacctagtcctgagcgc

SEQ ID NO: 288 - DNA, 22 bp, Artificial Sequence
  Description of Artificial Sequence: Synthetic oligonucleotide
tctgcacctagtcctgagcgca

SEQ ID NO: 289 - DNA, 20 bp, Artificial Sequence
  Description of Artificial Sequence: Synthetic oligonucleotide
tctgcacctagtcctgagcg

SEQ ID NO: 290 - DNA, 19 bp, Artificial Sequence
  Description of Artificial Sequence: Synthetic oligonucleotide
tctgcacctagtcctgagc

SEQ ID NO: 291 - DNA, 24 bp, Artificial Sequence
  Description of Artificial Sequence: Synthetic oligonucleotide
tctgcacctagtcctgagcgcatt

SEQ ID NO: 292 - DNA, 16 bp, Artificial Sequence
  Description of Artificial Sequence: Synthetic oligonucleotide
tctgcacctagtcctg

SEQ ID NO: 293 - DNA, 24 bp, Artificial Sequence
  Description of Artificial Sequence: Synthetic oligonucleotide
tctgcacctagtcctgagcgcaat

SEQ ID NO: 294 - DNA, 18 bp, Artificial Sequence
  Description of Artificial Sequence: Synthetic oligonucleotide
tctgcacctagtcctgag

SEQ ID NO: 295 - DNA, 23 bp, Artificial Sequence
  Description of Artificial Sequence: Synthetic oligonucleotide
tctgcacctagtcctgagcgcag

SEQ ID NO: 296 - DNA, 20 bp, Artificial Sequence
  Description of Artificial Sequence: Synthetic oligonucleotide
ctgcacctagtcctgagcgc

SEQ ID NO: 297 - DNA, 32 bp, Artificial Sequence
  Description of Artificial Sequence: Synthetic oligonucleotide
tagagtttctccagggtactgtgcgcagtgcg

SEQ ID NO: 298 - DNA, 22 bp, Artificial Sequence
  Description of Artificial Sequence: Synthetic oligonucleotide
gtttctccagggtactgtgcgc

SEQ ID NO: 299 - DNA, 19 bp, Artificial Sequence
  Description of Artificial Sequence: Synthetic oligonucleotide
gtttctccagggtactgtg

SEQ ID NO: 300 - DNA, 32 bp, Artificial Sequence
  Description of Artificial Sequence: Synthetic oligonucleotide
tagaggtttctccagggtactggcgcagtgcg

SEQ ID NO: 301 - DNA, 21 bp, Artificial Sequence
  Description of Artificial Sequence: Synthetic oligonucleotide
tttctccagggtactggcgca

SEQ ID NO: 302 - DNA, 22 bp, Artificial Sequence
  Description of Artificial Sequence: Synthetic oligonucleotide
gtttctccagggtactggcgca

SEQ ID NO: 303 - DNA, 20 bp, Artificial Sequence
  Description of Artificial Sequence: Synthetic oligonucleotide
gtttctccagggtactggcg

SEQ ID NO: 304 - DNA, 19 bp, Artificial Sequence
  Description of Artificial Sequence: Synthetic oligonucleotide
tttctccagggtactggcg

SEQ ID NO: 305 - DNA, 20 bp, Artificial Sequence
  Description of Artificial Sequence: Synthetic oligonucleotide
tttctccagggtactggcgc

SEQ ID NO: 306 - DNA, 21 bp, Artificial Sequence
  Description of Artificial Sequence: Synthetic oligonucleotide
gtttctccagggtactggcgc

SEQ ID NO: 307 - DNA, 19 bp, Artificial Sequence
  Description of Artificial Sequence: Synthetic oligonucleotide
gtttctccagggtactggc

SEQ ID NO: 308 - DNA, 22 bp, Artificial Sequence
  Description of Artificial Sequence: Synthetic oligonucleotide
tttctccagggtactggcgcag

SEQ ID NO: 309 - DNA, 18 bp, Artificial Sequence
  Description of Artificial Sequence: Synthetic oligonucleotide
gtttctccagggtactgg

SEQ ID NO: 310 - DNA, 23 bp, Artificial Sequence
  Description of Artificial Sequence: Synthetic oligonucleotide
tttctccagggtactggcgcatt

SEQ ID NO: 311 - DNA, 32 bp, Artificial Sequence
  Description of Artificial Sequence: Synthetic oligonucleotide
tagagtttgagctgcctggagggcgcagtgcg

SEQ ID NO: 312 - DNA, 22 bp, Artificial Sequence
  Description of Artificial Sequence: Synthetic oligonucleotide
tttgagctgcctggagggcgca

SEQ ID NO: 313 - DNA, 20 bp, Artificial Sequence
  Description of Artificial Sequence: Synthetic oligonucleotide
tttgagctgcctggagggcg

SEQ ID NO: 314 - DNA, 21 bp, Artificial Sequence
  Description of Artificial Sequence: Synthetic oligonucleotide
tttgagctgcctggagggcgc

SEQ ID NO: 315 - DNA, 19 bp, Artificial Sequence
  Description of Artificial Sequence: Synthetic oligonucleotide
tttgagctgcctggagggc

SEQ ID NO: 316 - DNA, 17 bp, Artificial Sequence
  Description of Artificial Sequence: Synthetic oligonucleotide
tttgagctgcctggagg

SEQ ID NO: 317 - DNA, 24 bp, Artificial Sequence
  Description of Artificial Sequence: Synthetic oligonucleotide
tttgagctgcctggagggcgcatt

SEQ ID NO: 318 - DNA, 18 bp, Artificial Sequence
  Description of Artificial Sequence: Synthetic oligonucleotide
tttgagctgcctggaggg

SEQ ID NO: 319 - DNA, 24 bp, Artificial Sequence
  Description of Artificial Sequence: Synthetic oligonucleotide
tttgagctgcctggagggcgcaat

SEQ ID NO: 320 - DNA, 16 bp, Artificial Sequence
  Description of Artificial Sequence: Synthetic oligonucleotide
tttgagctgcctggag

SEQ ID NO: 321 - DNA, 23 bp, Artificial Sequence
  Description of Artificial Sequence: Synthetic oligonucleotide
tttgagctgcctggagggcgcag

SEQ ID NO: 322 - RNA, 54 nt, Artificial Sequence
  Description of Artificial Sequence: Synthetic oligonucleotide
  modified_base (3)..(23): a, c, u, g, unknown or other
  modified_base (30)..(50): a, c, u, g, unknown or other
ggnnnnnnnnnnnnnnnnnnnnncucgagnnnnnnnnnnnnnnnnnnnnnuuuu

SEQ ID NO: 323 - RNA, 104 nt, Artificial Sequence
  Description of Artificial Sequence: Synthetic polynucleotide
  modified_base (25)..(45): a, c, u, g, unknown or other
  modified_base (61)..(81): a, c, u, g, unknown or other
ccuggccuccugcagugccacgcunnnnnnnnnnnnnnnnnnnnncuccaugugguagagnnnnnnnnnnnnnnnnnnnnnagugcggcacaugcuuaccagcu

SEQ ID NO: 324 - DNA, 31 bp, Artificial Sequence
  Description of Artificial Sequence: Synthetic oligonucleotide
tagagtctgtgcgtgttgcaagagaaagtgc

SEQ ID NO: 325 - DNA, 23 bp, Artificial Sequence
  Description of Artificial Sequence: Synthetic oligonucleotide
gacattctgcacctagtcctgat